European Patent Specification EP 2 652 133 B1, published May 10, 2023. Title: LIGATION METHOD EMPLOYING EUKARYOTIC tRNA LIGASE. Applicant: Ach, Robert Zeiner, Gusti. The sequence listing filed with the application follows.

SEQUENCE LISTING (7 sequences)

SEQ ID NO: 1 - DNA, 20 bp, Synthetic oligonucleotide
cagggtaatatagacacgtc

SEQ ID NO: 2 - DNA, 20 bp, Artificial Sequence
  Synthetic oligonucleotide
cagggtaatatagacacgtc

SEQ ID NO: 3 - DNA, 55 bp, Artificial Sequence
  Synthetic oligonucleotide
tgaactccatgcactacaagttaccgtaggcataacagggtaatatagacacgtc

SEQ ID NO: 4 - DNA, 55 bp, Artificial sequence; identical to SEQ ID NO: 3
  Synthetic oligonucleotide

SEQ ID NO: 5 - DNA, 55 bp, Artificial sequence; identical to SEQ ID NO: 3
  Synthetic oligonucleotide

SEQ ID NO: 6 - DNA, 33 bp, Artificial sequence
  Synthetic oligonucleotide
tgaactccatgcactacaagttaccgtaggcat

SEQ ID NO: 7 - DNA, 22 bp, Artificial sequence
  Synthetic oligonucleotide
aacagggtaatatagacacgtc